European Patent Specification EP 3 681 504 B1, published August 23, 2023. Title: METHODS OF DETECTION USING X-RAY FLUORESCENCE. Applicant: ICAGEN, Inc. WARNER, Benjamin P. HSIEH, Chang-Tai SOLOMON, Emilia PETERSON, Lori KRAFTE, Douglas ZAHLER, Nathan. The sequence listing filed with the application follows.

SEQUENCE LISTING (16 sequences)

SEQ ID NO: 1 - protein, 10 aa, Artificial Sequence
  Synthetic Peptide
  4-iodophenylalanine (1)..(1)
  4-bromophenylalanine (10)..(10)
FCDICPNHCF

SEQ ID NO: 2 - protein, 10 aa, Artificial Sequence
  Synthetic Peptide
  4-iodophenylalanine (1)..(1)
  4-bromophenylalanine (10)..(10)
FCQRCERWCF

SEQ ID NO: 3 - protein, 10 aa, Artificial Sequence
  Synthetic Peptide
  4-iodophenylalanine (1)..(1)
  4-bromophenylalanine (10)..(10)
FCFHCFSECF

SEQ ID NO: 4 - protein, 10 aa, Artificial Sequence
  Synthetic Peptide
  4-iodophenylalanine (1)..(1)
  4-bromophenylalanine (10)..(10)
FCAGCFTGCF

SEQ ID NO: 5 - protein, 10 aa, Artificial Sequence
  Synthetic Peptide
  4-iodophenylalanine (1)..(1)
  4-bromophenylalanine (10)..(10)
FCQLCNVLCF

SEQ ID NO: 6 - protein, 9 aa, Artificial Sequence
  Synthetic Peptide
  4-iodophenylalanine (1)..(1)
FCDICPNHC

SEQ ID NO: 7 - protein, 9 aa, Artificial Sequence
  Synthetic Peptide
  4-iodophenylalanine (1)..(1)
FCQRCERWC

SEQ ID NO: 8 - protein, 9 aa, Artificial Sequence
  Synthetic Peptide
  4-iodophenylalanine (1)..(1)
FCHTCFQTC

SEQ ID NO: 9 - protein, 6 aa, Artificial Sequence
  Synthetic Peptide
  3,5-dibromotyrosine (1)..(1)
  MISC_FEATURE (4)..(4): Xaa can be Glutamine (Q) or Threonine (T)
YCRXSC

SEQ ID NO: 10 - protein, 6 aa, Artificial Sequence
  Synthetic Peptide
  3,5-dibromotyrosine (1)..(1)
YCRTSC

SEQ ID NO: 11 - protein, 6 aa, Artificial Sequence
  Synthetic Peptide
  3,5-dibromotyrosine (1)..(1)
YCRQSC

SEQ ID NO: 12 - protein, 6 aa, Artificial Sequence
  Synthetic Sequence
  mono-iodo tyrosine (1)..(1)
  MISC_FEATURE (4)..(4): Xaa can be Glutamine (Q) or Threonine (T)
YCRXSC

SEQ ID NO: 13 - protein, 6 aa, Artificial Sequence
  Synthetic Sequence
  mono-iodo tyrosine (1)..(1)
YCRTSC

SEQ ID NO: 14 - protein, 6 aa, Artificial Sequence
  Synthetic Sequence
  mono-iodo tyrosine (1)..(1)
YCRQSC

SEQ ID NO: 15 - protein, 5 aa, Artificial Sequence
  Synthetic Sequence
CRTSC

SEQ ID NO: 16 - protein, 5 aa, Artificial Sequence
  Synthetic Sequence
CRQSC